European Patent Application EP 4 772 618 A1, published July 8, 2026. Title: 修饰的RNA去甲基化酶及其编码核酸、应用及植物培育方法、产物. Applicant: 超级植物（北京）科技有限公司. Application CN. The sequence listing filed with the application follows.

SEQUENCE LISTING (48 sequences)

SEQ ID NO: 1 - protein, 419 aa, Ostreococcus lucimarinus
MSPSSSVLEPEDGEPFARVHRAHYRGFVVDAPSVLPASLHDDVERAFDDMRSRGEFTHDVVSAGNKVSTTYVRRCLLGEDGMTYHYQKLRLFAQPWRGREAYEVVRRLNETLTRSARERCEKLGGAFAESECEYNVTLINYMETEGESEIELRNEEKFDLGTTSVSWHSDSSLRENSTVAVYHTYEAPERKDWRVALRALNAECEVLCVPLEDKATYYMCGEFNATHHHAVLTGSSARYSSTHRVAVVAKDTFQYIKRRCIDALAIVPDLERENKPLDAKQIQFLADVHREVEFQWIRMFHLQGEAHAAWHDTYWTRKIAELTEAWDRMEACFRVILSKLKRSSRSPESPPRAYAMLLYALKTVKELRDEYTKRTKASAYASLPPSQRPVDLPAYDNTSPLPFELKPVIYFLEEEQNKV

SEQ ID NO: 2 - protein, 522 aa, Aphanomyces astaci
MDPKERKKLERQKKKAKALERKSAKKPNVASLKPVSQPTTSHKRPSEPSGSSAAPPAKKQQIEKAKPLPVPSNYTGPEKFLTPSHPDFHDILTRSYVGFVHEPAAAQPREFHAGMRAAFEHLRDKGYFQYDVVMAGGKHLSRTFVRRTLVGNFGITYKYLGLRIFAHAWDVPSSAAVFRNLYALNQAIVARTKASASPAPPSCEYNLTLINYMEPDNPVLGLKDDLTYDMGKVSVSWHADSSLEDFSSIGVYHTLLPTKKSKKGPCDWRIAMRLSPDVPGAKTTPPLVVPTGDGDVYYLNGDFNHHHQHMVLSGTAVRVSSTHRVAVTAEDTLQYIQAKVTAALKSSAKDPQDKCRRGHADDVRHEQTTVTTLEMDWLRQYWIQGDKHNDLHVDWQQPMLALEASWRKLEARTKTLADALVQSHDVDDLKVLKAVLEGLRNRQVGRDQFVHRMKDKVFKRIAADFQPMERPVWTDWDDVHLLPKDLTATIAALHAHKLVLESEKKRQWKIHAGTRHNKINKA

SEQ ID NO: 3 - protein, 520 aa, Micromonas commode
MGKKHKPRPDDRARVVDASDVGGKVKKKKANGATMKASRRKGGGASANGDGRPYDPSRTLSKPAPPPPAYTPRVPTGAYITPEHDEYDACVARSYVGFVVDPPDILPDELHADVAAAFKTMAKRGLFTRDVLAAGKTVSPTFVSRTLVGERGMTYHYQKLRIFALPWSDEDTPEGSPLRVVRRLNDAMKRRSRALLTRHRDARVPGDVTGSCEFNVTLINLMEPERKESVALKDEGQFGMGKASVSWHSDSSLQDTSTVAVYHQTSGGIDGDDTSWHVALKCLDGVTPALRVPLRSHSAYYIMRDFNLHHHHAVLNGDTRRFSSTHRVAVTAKDTFDYVRGRCERALAVLPSLKWRAGRWPKGTKPPRDASSTQLSDAVRVLGETHREVEFQWIRMFWLQGTRHAAQHDGYWTRRIEELTQAWDVMELGLRFAMDACARAADGKAKAEPRAFEMLRYLLETIAELREEHDARTQSGAYAQVPDDCKPVDLPGFDDSSPLPRNLRPVLNTLERHRRRALDR

SEQ ID NO: 4 - protein, 541 aa, Micromonas pusilla
MATATGSSGGKLEKRKKKKKKTTAVERAGSGGGGNAKKPTTTTASHRPTKPLLRAAPPPPSYRLRGTSGSDDDDDDAAPSFLTPSHAEYERCMKTSYLGFHVDDPSALPEKTHREIARAFERMASDGIFHRDVLAAGKSVSPTFVSRTLLGERGMTYHYQRLRIFAHPWDEETQPDASHPFRAVKRLNDALVSRSTAVLRASSDPRLGDGVDGSCDFNVTLINLMEPASRCAEVPLKDEALFGMGKARSTSVSWHSDSSLQDVSTVAVYHQTDDDDDDSWAVALKTLDGVTPAMRTPLRSREMYYMLRDFNAHHHHAVITGESRRFSSTHRVAVVAKDTFEHIKTRCERALRLLPGIKKIAQVGPGPGDDLAAFARSAQMMGETHRECEFQWIRMFWLQGSRHAASHSAYWRQRIAELTQAWDAMELGYRWALDALRAGASTGAMPLRAYDVVSYLLEETRELRAEHARRSRAGAYEAMPADCRPVDEPKFDEKSPLPFDLGPVLATLAGWRRDAERAQTTTTEGGSKTKKGKPGKGSKRR

SEQ ID NO: 5 - protein, 506 aa, Polarella glacialis
MDMDRFVREPADASSESFHEEFRRCLHGLYEQGIFQYDLIQPVGPGTPVVSTRVTRCLIGEPGITYKYLGLRMFAHPWKGEKTSESCSAMYQHNQELISKAEEQAVAVGCDAPPYSSCFNLTLINRMDPADSGAPNKLGAVSVSWHADSSLVDYSTITVYVAEHDATQDSFGLSPARPCKPCDDPWRVALRHTPNVQGPEKSCPWEVAAQETAKPVKRRAKAKVHTVPIHDGDIYHLIGDFNHHNQHAVLAGRDAVLAVRRGMPVLGGSGTIRYSSTHRVALTEGHSYRSVKQRCSTALSVALADMIPAAAQVHEEQQCSLELEFEWIRQFFIQGKAHREALPWWHSKMDELVFLWRQFEVLTAQRLTLLRRAAAGKVGTSELDPFCLALKNGLQKRAELREAWRQREHDPLLKKQPANRQPLQCLFDAPSDAPHGAGSEALPHNVWPLVEEISQIQLQLHETKKVGKPWYQFVLNVYQGCAFQGGEVTCLSWTLFSQRLPMKRRW

SEQ ID NO: 6 - protein, 543 aa, Guillardia theta
MQETLWQRVKEGLEWFDGAIGEGEEEEEAGRIAGNKGGGRRRGFEQALERYYPKFRVIHRDLLPSALEPSTRRALEVLKDQMGWFRRDYVWVKGKVTQTMVTRLLVGERGCTYKYKGLRLFCRSWETEAAKVPDSACHALAEIRRLNEVLKEKSRKQHECFMARGEGSGEGAVEGGVNSFNATLINYFDESIANHVETRPEPYYGMGRCCISWHADDGVVEQSAIAVYNVIERAEKGEEEELGEVWKVGLKVKWEVDTPGVAVPMVNGDAYVMLSGFNEKNQHCVVCGRGSRFSSTHRVCPQEDMYHNFYCRCRETFLQLHFPWNARGVLQEGEERRACLSKIVASLDALEDLHDQLEFEWLRQFHFQYFDLPPSELDDYWVEVIHVLADLWQRMEIVVWIWISCCRRKSFMVGGKELRDRLERLRQLTSQQKGQGQEVQSSLPFLMKKLLRSEGAGGGREAAGEKAIPEDALELVKATLARRLQKRQEHRIWWEENFRKRLSMGRGGEQREGGKRKRKEGRADGLGFSLLPANLNSLVSTLK

SEQ ID NO: 7 - protein, 420 aa, Ostreococcus tauri
MPDVLGPGDGDAYERVRSFHYDGFVVDDPEILPEALHDDVARAFDSLLREGEFTHDVLSAGNKVSRTFVTRTLLGDRGTTYHYQKLRLFAQPWDGEKRWEYATARRLNEALTRRTREILRGTRHGESECEYNVTLINRMDTREESEVALKDEALFDLGTTSVSWHSDSSLRENSTVAVYSTVDDPERADWSVALRALGKQCPALRVPLKDKATYYMCGDFNATHHHAVLTGSSARYSSTHRVGVVEKDTFQYIKRRCLEALALIPDLENKSASLDAKKIQLLAEIHREVEFQWIRMFHLQGDTHARQHKTYWTQRIAELTEAWDRMEACFRAILSKLKLSPESTPQPSRAYSMMLYAMKEVKELRDEHVKRISASAYAALPESQRPVDLPQYDDTSPLPFELKPVIYFVEAEQAKLKGES

SEQ ID NO: 8 - protein, 787 aa, Ectocarpus sp
MTMTTATTVATTSRLLSPPTSEATTPIQHSNSGMEVSTEKTSHKKKRKSKRKRQQQERDTSSIPDASRQSRGSSSSSTRPPPPPPPPPPTTTTTTTSKKHSRIKEKPARFVHPHLDAELRRLGRSWLSPGDPLFKPALDRSYRGVRHEPGGSLPQAVHRGFRQSFDSLHEAGLFLYDTVQAGGKRLSRTFVTRTLVGDAGITYKYLGLRLFAHPWGLGESDFRKGPGDSLADALNDPCLADLFSNDGSGFDDNDRVADTLRKVGDLSEWMRLRAGAMLKEEVGEAGGERGSCAFNLTLINRMECSGAKRDLKPDPLFSMGKFSVSWHADSCLQDFSTIGVYHCTDPVPAEPDWGIALRVSTEARVGGGGGGSGDGDGYGVSNVEKTRRKEAERGVKPAGPKAIASVAASAAGAVPEKQGEQVLTPPLLIPLQSGDAYFLLDDFNHFHEHAVVSGSSTLRYSSTHRVADTDGNTFSHVQKRCERALAGGGSAAAGGDYHILNLAQVRAEQALLTELESEWLNQFWVQGRRHASLHPWWRGPMALVLATWRELERRTALTVRRLMSLRGQGGGEGVGPGGGGTAAETAGAEPAAIAKAFETVLRALEVRRESRSRWGARFADSAYRSLAADLAPVVPALWPAEGSSGGDVGEEGSPLLLPQSLGGIVSRLRECYTVVYRAASGGKKAGSAKAIAAGAASNWELFRAASSSSSSGGGGAGKKHGSALGKQQQQQQQQQQQQRKMRGLAGQDGLEKTKKRAGGVVKGGGDGGGGRTLKGQGSRRKDRVRER

SEQ ID NO: 9 - protein, 715 aa, Conferva siliculosa
MTTTSATTAARSRLPSPPTSAATTPIQHSNNGTEASPEKTSNKKKAKNKRKRQQECSIPAASQQSRGSSSSSTRPPPPTTTTLKKHSRIKEKPARFVHPHLDAELRRLGRSWLSPGDPLFTPALDRSYRGVRHEPAGSLPQAVHSGFRQSFDSLHEAGLFLYDTVQAGGKRLSRTFVTRTLVGDAGITYKYLGLRLFAHPWGLGESDFRKGPGDGLADALNDPCLADLFSKDGASSVRKSKDNLRGSRFDDNDRVADTLRKVGDLSEWMRLRAGAMLKEEVREAGGERGSCAFNLTLINRMECSGAKRDLKPDPLFSMGKCSVSWHADSCLQDFSTIGVYHCTDPVPAEPDWGIALRVSTEARVGGDGGGDGDGNGVSNDEKTRRKEAERGLKPAGPKAVASVAASAAEAVPEKQGEQVLTPPLLIPLQSGDAYFLLDDFNHFHEHAVVSGSSTLRYSSTHRVADTDGNTFSHVQKRCEQALAGGGSAAAGGDDQILNLAQVRAEQALLTELESEWLNQFWVQGRRHASLHPWWRGPMALVLATWRELERRTSLTVQHLMSLRGQDGGEALWPAEGSGGGDVGEEGSTLLLPQSLGGVISRLRECYTVVYRAASGGKKAGSAKAIAAGAASNWELFRAASSSASSGGGGAGKKHGSALGKQQQQQQQRKKRGAAGQDGLEKKKRAGGVVKGGGDGGGGRTSKGQRSRRKGRVRER

SEQ ID NO: 10 - protein, 417 aa, Fragilariopsis cylindrus
MLTPEDGVYFQKHLQDHYKGFVHLPVDRLEPRDFHEEFKNSLERLRDAGYYQYDVVMAGGKYSSRTFVKRTLVGNPGITYKYLGLRLFAHAWSGPGCTPLMKSIGDMNQSMIKMTEQFPENERCDYNLTLINYMEPTTHTKVGFKDEANYGMGKVSVSWHADSSLVDNSSIGVYHCLPTQRNSKWDWKIALRPLAIESKDNTGSTKRDNKSTTPKPVVVNTKDGDAYFLLGNFNMKHQHCVLAGSQANRISSTHRVAVTIEDTYDYILKRVKIARKRFRLQMETIPPSLQSPVVGLDAKVIRYCQRILTEVEMEWIAQYWLQGDQHDKMRVWWQKPMKTLEAYWCALEVYTYRLFEFLLSRIASNDTVPIDVVKVLIIEFKTRQSFREQWDERRSDKIYQRRVSEEFRPVARPIFEN

SEQ ID NO: 11 - protein, 528 aa, Acanthaster planci
MRFLSLNVLRRWMSKMSKRRQTEDLGKEVKKKKLLSEVARGRLQFLMPDHPDFKSLMRKSYFNFAHEPSTGIPVSLHEELTWALDILRYHGYFYRDWVKVKGQTVQTPISRTLIGEPGTTYKYLGLRLFTIPWSFGHHKPESEVELASETIGKLNEHYKAVSRRLLRKKTAEQTHLKSSPSQEVAPCSSKDRPRERICVEEPKQMTHGLSIEEGTNFNVVLINYMDPEDPDLRLKPEPYYGMGPLAVSWHMDGNLVRGSTVAVYNHTCSSDGGDSTTDSDWMVGFKVSWDIETPGVAIPLQTGESYFMLGDLNDTHQHCVVAGSQARFSTTHRVADCQQGTLSYIQQRCLEALGNLSQLENGEYELKSFQAGHLDFTETVHNEVEFEWLRQFWMQGSRHAAERGGWVPAMECLEADWNKMEHMTKLAVEEANRLGPEEGSVIAEALLPHLKERRKLRQECLDKFPRRLLETIHRDFLPIHRPKWDNDDPSQPLPFDLKGIIRKMRLLCNGKRIKSPSDSESSDTGLHS

SEQ ID NO: 12 - protein, 485 aa, Saccoglossus kowalevskii
MNPRMKRKIPRIPLVTSEGEVAGQLALPIRKQKLLSAVKETQVKFLSPVDTDYKALVAENYDNFVVQPGTELSSELHTRLQQGFETLLTNGYLYQHRIRFRNKTVMTPVSRTLIGEPGMTYRYLNLRLFALPWTFDDKKKLSDVEKACNAFYELNTYFKDHVNKLITEKFASSTGRKIDETDDSLKTIIQRNTEFKATILNYMDPSEIRLKQEPYYNMGDIAVSWHKDESLVDGSTVAVYNHVPMEARQDCSKWKVGLKVAWDITTPAVCTPLNNKDCYYMLDTMNDTHQHCVIAGTLPRYSSTHRVVESSDSTLCYIQQRCQTALDNIGYKDQIPYLKSLETDVLQLIEEIHSEIEFEWLRQFWMQGTQHSQERQYWLKPMEQLQEDWKTMELMTKLMIDIVVKKKDQSHMIAKILLPSLVERNELRNEWMNRYSEKEFYHIPEEHRPIYEPCWTDANSEMPLPFDLSQHIDIIQECMDTNDSQ

SEQ ID NO: 13 - protein, 423 aa, Ostreococcus lucimarinus
MRPRKSPSSSVLEPEDGEPFARVHRAHYRGFVVDAPSVLPASLHDDVERAFDDMRSRGEFTHDVVSAGNKVSTTYVRRCLLGEDGMTYHYQKLRLFAQPWRGREAYEVVRRLNETLTRSARERCEKLGGAFAESECEYNVTLINYMETEGESEIELRNEEKFDLGTTSVSWHSDSSLRENSTVAVYHTYEAPERKDWRVALRALNAECEVLCVPLEDKATYYMCGEFNATHHHAVLTGSSARYSSTHRVAVVAKDTFQYIKRRCIDALAIVPDLERENKPLDAKQIQFLADVHREVEFQWIRMFHLQGEAHAAWHDTYWTRKIAELTEAWDRMEACFRVILSKLKRSSRSPESPPRAYAMLLYALKTVKELRDEYTKRTKASAYASLPPSQRPVDLPAYDNTSPLPFELKPVIYFLEEEQNKV

SEQ ID NO: 14 - protein, 426 aa, Ostreococcus lucimarinus
MSPSSSVLEPEDGEPFARVHRAHYRGFVVDAPSVLPASLHDDVERAFDDMRSRGEFTHDVVSAGNKVSTTYVRRCLLGEDGMTYHYQKLRLFAQPWRGREAYEVVRRLNETLTRSARERCEKLGGAFAESECEYNVTLINYMETEGESEIELRNEEKFDLGTTSVSWHSDSSLRENSTVAVYHTYEAPERKDWRVALRALNAECEVLCVPLEDKATYYMCGEFNATHHHAVLTGSSARYSSTHRVAVVAKDTFQYIKRRCIDALAIVPDLERENKPLDAKQIQFLADVHREVEFQWIRMFHLQGEAHAAWHDTYWTRKIAELTEAWDRMEACFRVILSKLKRSSRSPESPPRAYAMLLYALKTVKELRDEYTKRTKASAYASLPPSQRPVDLPAYDNTSPLPFELKPVIYFLEEEQNKVPKKKRKV

SEQ ID NO: 15 - protein, 479 aa, Ostreococcus lucimarinus
MKRTPTAEERERGAKKLRLLEELEDTWLPYLSPSSSVLEPEDGEPFARVHRAHYRGFVVDAPSVLPASLHDDVERAFDDMRSRGEFTHDVVSAGNKVSTTYVRRCLLGEDGMTYHYQKLRLFAQPWRGREAYEVVRRLNETLTRSARERCEKLGGAFAESECEYNVTLINYMETEGESEIELRNEEKFDLGTTSVSWHSDSSLRENSTVAVYHTYEAPERKDWRVALRALNAECEVLCVPLEDKATYYMCGEFNATHHHAVLTGSSARYSSTHRVAVVAKDTFQYIKRRCIDALAIVPDLERENKPLDAKQIQFLADVHREVEFQWIRMFHLQGEAHAAWHDTYWTRKIAELTEAWDRMEACFRVILSKLKRSSRSPESPPRAYAMLLYALKTVKELRDEYTKRTKASAYASLPPSQRPVDLPAYDNTSPLPFELKPVIYFLEEEQNKVKRTPTAEERERGAKKLRLLEELEDTWLPYL

SEQ ID NO: 16 - protein, 527 aa, Aphanomyces astaci
MRKVIKDPKERKKLERQKKKAKALERKSAKKPNVASLKPVSQPTTSHKRPSEPSGSSAAPPAKKQQIEKAKPLPVPSNYTGPEKFLTPSHPDFHDILTRSYVGFVHEPAAAQPREFHAGMRAAFEHLRDKGYFQYDVVMAGGKHLSRTFVRRTLVGNFGITYKYLGLRIFAHAWDIPSSAAVFRNLYALNQAIVARTKASASPAPPSCEYNLTLINYMEPDNPVLGLKDDPTYDMGKVSVSWHADSSLEDFSSIGVYHTLLPTKKSKKGPCDWRIAMRLSPDVPGAKTTPPLVVPTGDGDVYYLNGDFNHHHQHMVLSGTAVRVSSTHRVAVTAEDTLQYIQAKVTASLKSSAKDPQDKCRRGHADDVRHEQTTVTTLEMDWLRQYWIQGDKHNDLHVDWQQPMLALEASWRKLEARTKTLADALVQSHDVDDLKVLKAVLEGLRNRQVGRDQFVHRMKDKVFKRIAADFQPMERPVWTDWDDVHLLPKDLTATIAALHAHKLVLESEKKRQWKIHAGTRHHKNNKA

SEQ ID NO: 17 - protein, 538 aa, Aphanomyces astaci
MDPKERKKLERQKKKAKALERKSAKKPNVASLKPVSQPTTSHKRPSEPSGSSAAPPAKKQQIEKAKPLPVPSNYTGPEKFLTPSHPDFHDILTRSYVGFVHEPAAAQPREFHAGMRAAFEHLRDKGYFQYDVVMAGGKHLSRTFVRRTLVGNFGITYKYLGLRIFAHAWDIPSSAAVFRNLYALNQAIVARTKASASPAPPSCEYNLTLINYMEPDNPVLGLKDDPTYDMGKVSVSWHADSSLEDFSSIGVYHTLLPTKKSKKGPCDWRIAMRLSPDVPGAKTTPPLVVPTGDGDVYYLNGDFNHHHQHMVLSGTAVRVSSTHRVAVTAEDTLQYIQAKVTASLKSSAKDPQDKCRRGHADDVRHEQTTVTTLEMDWLRQYWIQGDKHNDLHVDWQQPMLALEASWRKLEARTKTLADALVQSHDVDDLKVLKAVLEGLRNRQVGRDQFVHRMKDKVFKRIAADFQPMERPVWTDWDDVHLLPKDLTATIAALHAHKLVLESEKKRQWKIHAGTRHHKNNKAKRPAATKKAGQAKKKK

SEQ ID NO: 18 - protein, 582 aa, Aphanomyces astaci
MKRTPTAEERERGAKKLRLLEELEDTWLPYLDPKERKKLERQKKKAKALERKSAKKPNVASLKPVSQPTTSHKRPSEPSGSSAAPPAKKQQIEKAKPLPVPSNYTGPEKFLTPSHPDFHDILTRSYVGFVHEPAAAQPREFHAGMRAAFEHLRDKGYFQYDVVMAGGKHLSRTFVRRTLVGNFGITYKYLGLRIFAHAWDIPSSAAVFRNLYALNQAIVARTKASASPAPPSCEYNLTLINYMEPDNPVLGLKDDPTYDMGKVSVSWHADSSLEDFSSIGVYHTLLPTKKSKKGPCDWRIAMRLSPDVPGAKTTPPLVVPTGDGDVYYLNGDFNHHHQHMVLSGTAVRVSSTHRVAVTAEDTLQYIQAKVTASLKSSAKDPQDKCRRGHADDVRHEQTTVTTLEMDWLRQYWIQGDKHNDLHVDWQQPMLALEASWRKLEARTKTLADALVQSHDVDDLKVLKAVLEGLRNRQVGRDQFVHRMKDKVFKRIAADFQPMERPVWTDWDDVHLLPKDLTATIAALHAHKLVLESEKKRQWKIHAGTRHHKNNKAKRTPTAEERERGAKKLRLLEELEDTWLPYL

SEQ ID NO: 19 - protein, 526 aa, Micromonas commode
MRNKKKKGKKHKPRPDDRARVVDASDVGGKVKKKKANGATMKASRRKGGGASANGDGRPYDPSRTLSKPAPPPPAYTPRVPTGAYITPEHDEYDACVARSYVGFVVDPPDILPDELHADVAAAFKTMAKRGLFTRDVLAAGKTVSPTFVSRTLVGERGMTYHYQKLRIFALPWSDEDTPEGSPLRVVRRLNDAMKRRSRALLTRHRDARVPGDVTGSCEFNVTLINLMEPERKESVALKDEGQFGMGKASVSWHSDSSLQDTSTVAVYHQTSGGIDGDDTSWHVALKCLDGVTPALRVPLRSHSAYYIMRDFNLHHHHAVLNGDTRRFSSTHRVAVTAKDTFDYVRGRCERALAVLPSLKWRAGRWPKGTKPPRDASSTQLSDAVRVLGETHREVEFQWIRMFWLQGTRHAAQHDGYWTRRIEELTQAWDVMELGLRFAMDACARAADGKAKAEPRAFEMLRYLLETIAELREEHDARTQSGAYAQVPDDCKPVDLPGFDDSSPLPRNLRPVLNTLERHRRRALDR

SEQ ID NO: 20 - protein, 547 aa, Micromonas commode
MGKKHKPRPDDRARVVDASDVGGKVKKKKANGATMKASRRKGGGASANGDGRPYDPSRTLSKPAPPPPAYTPRVPTGAYITPEHDEYDACVARSYVGFVVDPPDILPDELHADVAAAFKTMAKRGLFTRDVLAAGKTVSPTFVSRTLVGERGMTYHYQKLRIFALPWSDEDTPEGSPLRVVRRLNDAMKRRSRALLTRHRDARVPGDVTGSCEFNVTLINLMEPERKESVALKDEGQFGMGKASVSWHSDSSLQDTSTVAVYHQTSGGIDGDDTSWHVALKCLDGVTPALRVPLRSHSAYYIMRDFNLHHHHAVLNGDTRRFSSTHRVAVTAKDTFDYVRGRCERALAVLPSLKWRAGRWPKGTKPPRDASSTQLSDAVRVLGETHREVEFQWIRMFWLQGTRHAAQHDGYWTRRIEELTQAWDVMELGLRFAMDACARAADGKAKAEPRAFEMLRYLLETIAELREEHDARTQSGAYAQVPDDCKPVDLPGFDDSSPLPRNLRPVLNTLERHRRRALDRTLLLRETMNNLGVSDHAVLSRKTPQPY

SEQ ID NO: 21 - protein, 580 aa, Micromonas commode
MKRTPTAEERERGAKKLRLLEELEDTWLPYLGKKHKPRPDDRARVVDASDVGGKVKKKKANGATMKASRRKGGGASANGDGRPYDPSRTLSKPAPPPPAYTPRVPTGAYITPEHDEYDACVARSYVGFVVDPPDILPDELHADVAAAFKTMAKRGLFTRDVLAAGKTVSPTFVSRTLVGERGMTYHYQKLRIFALPWSDEDTPEGSPLRVVRRLNDAMKRRSRALLTRHRDARVPGDVTGSCEFNVTLINLMEPERKESVALKDEGQFGMGKASVSWHSDSSLQDTSTVAVYHQTSGGIDGDDTSWHVALKCLDGVTPALRVPLRSHSAYYIMRDFNLHHHHAVLNGDTRRFSSTHRVAVTAKDTFDYVRGRCERALAVLPSLKWRAGRWPKGTKPPRDASSTQLSDAVRVLGETHREVEFQWIRMFWLQGTRHAAQHDGYWTRRIEELTQAWDVMELGLRFAMDACARAADGKAKAEPRAFEMLRYLLETIAELREEHDARTQSGAYAQVPDDCKPVDLPGFDDSSPLPRNLRPVLNTLERHRRRALDRKRTPTAEERERGAKKLRLLEELEDTWLPYL

SEQ ID NO: 22 - protein, 545 aa, Micromonas pusilla
MRPRKATATGSSGGKLEKRKKKKKKTTAVERAGSGGGGNAKKPTTTTASHRPTKPLLRAAPPPPSYRLRGTSGSDDDDDDAAPSFLTPSHAEYERCMKTSYLGFHVDDPSALPEKTHREIARAFERMASDGIFHRDVLAAGKSVSPTFVSRTLLGERGMTYHYQRLRIFAHPWDEETQPDASHPFRAVKRLNDALVSRSTAVLRASSDPRLGDGVDGSCDFNVTLINLMEPASRCAEVPLKDEALFGMGKARSTSVSWHSDSSLQDVSTVAVYHQTDDDDDDSWAVALKTLDGVTPAMRTPLRSREMYYMLRDFNAHHHHAVITGESRRFSSTHRVAVVAKDTFEHIKTRCERALRLLPGIKKIAQVGPGPGDDLAAFARSAQMMGETHRECEFQWIRMFWLQGSRHAASHSAYWRQRIAELTQAWDAMELGYRWALDALRAGASTGAMPLRAYDVVSYLLEETRELRAEHARRSRAGAYEAMPADCRPVDEPKFDEKSPLPFDLGPVLATLAGWRRDAERAQTTTTEGGSKTKKGKPGKGSKRR

SEQ ID NO: 23 - protein, 557 aa, Micromonas pusilla
MATATGSSGGKLEKRKKKKKKTTAVERAGSGGGGNAKKPTTTTASHRPTKPLLRAAPPPPSYRLRGTSGSDDDDDDAAPSFLTPSHAEYERCMKTSYLGFHVDDPSALPEKTHREIARAFERMASDGIFHRDVLAAGKSVSPTFVSRTLLGERGMTYHYQRLRIFAHPWDEETQPDASHPFRAVKRLNDALVSRSTAVLRASSDPRLGDGVDGSCDFNVTLINLMEPASRCAEVPLKDEALFGMGKARSTSVSWHSDSSLQDVSTVAVYHQTDDDDDDSWAVALKTLDGVTPAMRTPLRSREMYYMLRDFNAHHHHAVITGESRRFSSTHRVAVVAKDTFEHIKTRCERALRLLPGIKKIAQVGPGPGDDLAAFARSAQMMGETHRECEFQWIRMFWLQGSRHAASHSAYWRQRIAELTQAWDAMELGYRWALDALRAGASTGAMPLRAYDVVSYLLEETRELRAEHARRSRAGAYEAMPADCRPVDEPKFDEKSPLPFDLGPVLATLAGWRRDAERAQTTTTEGGSKTKKGKPGKGSKRRKRPAATKKAGQAKKKK

SEQ ID NO: 24 - protein, 555 aa, Micromonas pusilla
MPKKKRKVATATGSSGGKLEKRKKKKKKTTAVERAGSGGGGNAKKPTTTTASHRPTKPLLRAAPPPPSYRLRGTSGSDDDDDDAAPSFLTPSHAEYERCMKTSYLGFHVDDPSALPEKTHREIARAFERMASDGIFHRDVLAAGKSVSPTFVSRTLLGERGMTYHYQRLRIFAHPWDEETQPDASHPFRAVKRLNDALVSRSTAVLRASSDPRLGDGVDGSCDFNVTLINLMEPASRCAEVPLKDEALFGMGKARSTSVSWHSDSSLQDVSTVAVYHQTDDDDDDSWAVALKTLDGVTPAMRTPLRSREMYYMLRDFNAHHHHAVITGESRRFSSTHRVAVVAKDTFEHIKTRCERALRLLPGIKKIAQVGPGPGDDLAAFARSAQMMGETHRECEFQWIRMFWLQGSRHAASHSAYWRQRIAELTQAWDAMELGYRWALDALRAGASTGAMPLRAYDVVSYLLEETRELRAEHARRSRAGAYEAMPADCRPVDEPKFDEKSPLPFDLGPVLATLAGWRRDAERAQTTTTEGGSKTKKGKPGKGSKRRPKKKRKV

SEQ ID NO: 25 - protein, 512 aa, Polarella glacialis
MRNKKKKDMDRFVREPADASSESFHEEFRRCLHGLYEQGIFQYDLIQPVGPGTPVVSTRVTRCLIGEPGITYKYLGLRMFAHPWKGEKTSESCSAMYQHNQELISKAEEQAVAVGCDAPPYSSCFNLTLINRMDPADSGAPNKLGAVSVSWHADSSLVDYSTITVYVAEHDATQDSFGLSPARPCKPCDDPWRVALRHTPNVQGPEKSCPWEVAAQETAKPVKRRAKAKVHTVPIHDGDIYHLIGDFNHHNQHAVLAGRDAVLAVRRGMPVLGGSGTIRYSSTHRVALTEGHSYRSVKQRCSTALSVALADMIPAAAQVHEEQQCSLELEFEWIRQFFIQGKAHREALPWWHSKMDELVFLWRQFEVLTAQRLTLLRRAAAGKVGTSELDPFCLALKNGLQKRAELREAWRQREHDPLLKKQPANRQPLQCLFDAPSDAPHGAGSEALPHNVWPLVEEISQIQLQLHETKKVGKPWYQFVLNVYQGCAFQGGEVTCLSWTLFSQRLPMKRRW

SEQ ID NO: 26 - protein, 533 aa, Polarella glacialis
MDMDRFVREPADASSESFHEEFRRCLHGLYEQGIFQYDLIQPVGPGTPVVSTRVTRCLIGEPGITYKYLGLRMFAHPWKGEKTSESCSAMYQHNQELISKAEEQAVAVGCDAPPYSSCFNLTLINRMDPADSGAPNKLGAVSVSWHADSSLVDYSTITVYVAEHDATQDSFGLSPARPCKPCDDPWRVALRHTPNVQGPEKSCPWEVAAQETAKPVKRRAKAKVHTVPIHDGDIYHLIGDFNHHNQHAVLAGRDAVLAVRRGMPVLGGSGTIRYSSTHRVALTEGHSYRSVKQRCSTALSVALADMIPAAAQVHEEQQCSLELEFEWIRQFFIQGKAHREALPWWHSKMDELVFLWRQFEVLTAQRLTLLRRAAAGKVGTSELDPFCLALKNGLQKRAELREAWRQREHDPLLKKQPANRQPLQCLFDAPSDAPHGAGSEALPHNVWPLVEEISQIQLQLHETKKVGKPWYQFVLNVYQGCAFQGGEVTCLSWTLFSQRLPMKRRWTLLLRETMNNLGVSDHAVLSRKTPQPY

SEQ ID NO: 27 - protein, 539 aa, Polarella glacialis
MKRPAATKKAGQAKKKKMDMDRFVREPADASSESFHEEFRRCLHGLYEQGIFQYDLIQPVGPGTPVVSTRVTRCLIGEPGITYKYLGLRMFAHPWKGEKTSESCSAMYQHNQELISKAEEQAVAVGCDAPPYSSCFNLTLINRMDPADSGAPNKLGAVSVSWHADSSLVDYSTITVYVAEHDATQDSFGLSPARPCKPCDDPWRVALRHTPNVQGPEKSCPWEVAAQETAKPVKRRAKAKVHTVPIHDGDIYHLIGDFNHHNQHAVLAGRDAVLAVRRGMPVLGGSGTIRYSSTHRVALTEGHSYRSVKQRCSTALSVALADMIPAAAQVHEEQQCSLELEFEWIRQFFIQGKAHREALPWWHSKMDELVFLWRQFEVLTAQRLTLLRRAAAGKVGTSELDPFCLALKNGLQKRAELREAWRQREHDPLLKKQPANRQPLQCLFDAPSDAPHGAGSEALPHNVWPLVEEISQIQLQLHETKKVGKPWYQFVLNVYQGCAFQGGEVTCLSWTLFSQRLPMKRRWKRPAATKKAGQAKKKK

SEQ ID NO: 28 - protein, 550 aa, Guillardia theta
MPKKKRKVQETLWQRVKEGLEWFDGAIGEGEEEEEAGRIAGNKGGGRRRGFEQALERYYPKFRVIHRDLLPSALEPSTRRALEVLKDQMGWFRRDYVWVKGKVTQTMVTRLLVGERGCTYKYKGLRLFCRSWETEAAKVPDSACHALAEIRRLNEVLKEKSRKQHECFMARGEGSGEGAVEGGVNSFNATLINYFDESIANHVETRPEPYYGMGRCCISWHADDGVVEQSAIAVYNVIERAEKGEEEELGEVWKVGLKVKWEVDTPGVAVPMVNGDAYVMLSGFNEKNQHCVVCGRGSRFSSTHRVCPQEDMYHNFYCRCRETFLQLHFPWNARGVLQEGEERRACLSKIVASLDALEDLHDQLEFEWLRQFHFQYFDLPPSELDDYWVEVIHVLADLWQRMEIVVWIWISCCRRKSFMVGGKELRDRLERLRQLTSQQKGQGQEVQSSLPFLMKKLLRSEGAGGGREAAGEKAIPEDALELVKATLARRLQKRQEHRIWWEENFRKRLSMGRGGEQREGGKRKRKEGRADGLGFSLLPANLNSLVSTLK

SEQ ID NO: 29 - protein, 548 aa, Guillardia theta
MQETLWQRVKEGLEWFDGAIGEGEEEEEAGRIAGNKGGGRRRGFEQALERYYPKFRVIHRDLLPSALEPSTRRALEVLKDQMGWFRRDYVWVKGKVTQTMVTRLLVGERGCTYKYKGLRLFCRSWETEAAKVPDSACHALAEIRRLNEVLKEKSRKQHECFMARGEGSGEGAVEGGVNSFNATLINYFDESIANHVETRPEPYYGMGRCCISWHADDGVVEQSAIAVYNVIERAEKGEEEELGEVWKVGLKVKWEVDTPGVAVPMVNGDAYVMLSGFNEKNQHCVVCGRGSRFSSTHRVCPQEDMYHNFYCRCRETFLQLHFPWNARGVLQEGEERRACLSKIVASLDALEDLHDQLEFEWLRQFHFQYFDLPPSELDDYWVEVIHVLADLWQRMEIVVWIWISCCRRKSFMVGGKELRDRLERLRQLTSQQKGQGQEVQSSLPFLMKKLLRSEGAGGGREAAGEKAIPEDALELVKATLARRLQKRQEHRIWWEENFRKRLSMGRGGEQREGGKRKRKEGRADGLGFSLLPANLNSLVSTLKRKVIK

SEQ ID NO: 30 - protein, 551 aa, Guillardia theta
MRPRKQETLWQRVKEGLEWFDGAIGEGEEEEEAGRIAGNKGGGRRRGFEQALERYYPKFRVIHRDLLPSALEPSTRRALEVLKDQMGWFRRDYVWVKGKVTQTMVTRLLVGERGCTYKYKGLRLFCRSWETEAAKVPDSACHALAEIRRLNEVLKEKSRKQHECFMARGEGSGEGAVEGGVNSFNATLINYFDESIANHVETRPEPYYGMGRCCISWHADDGVVEQSAIAVYNVIERAEKGEEEELGEVWKVGLKVKWEVDTPGVAVPMVNGDAYVMLSGFNEKNQHCVVCGRGSRFSSTHRVCPQEDMYHNFYCRCRETFLQLHFPWNARGVLQEGEERRACLSKIVASLDALEDLHDQLEFEWLRQFHFQYFDLPPSELDDYWVEVIHVLADLWQRMEIVVWIWISCCRRKSFMVGGKELRDRLERLRQLTSQQKGQGQEVQSSLPFLMKKLLRSEGAGGGREAAGEKAIPEDALELVKATLARRLQKRQEHRIWWEENFRKRLSMGRGGEQREGGKRKRKEGRADGLGFSLLPANLNSLVSTLKRPRK

SEQ ID NO: 31 - protein, 454 aa, Ostreococcus tauri
MPKKKRKVTLLLRETMNNLGVSDHAVLSRKTPQPYPDVLGPGDGDAYERVRSFHYDGFVVDDPEILPEALHDDVARAFDSLLREGEFTHDVLSAGNKVSRTFVTRTLLGDRGTTYHYQKLRLFAQPWDGEKRWEYATARRLNEALTRRTREILRGTRHGESECEYNVTLINRMDTREESEVALKDEALFDLGTTSVSWHSDSSLRENSTVAVYSTVDDPERADWSVALRALGKQCPALRVPLKDKATYYMCGDFNATHHHAVLTGSSARYSSTHRVGVVEKDTFQYIKRRCLEALALIPDLENKSASLDAKKIQLLAEIHREVEFQWIRMFHLQGDTHARQHKTYWTQRIAELTEAWDRMEACFRAILSKLKLSPESTPQPSRAYSMMLYAMKEVKELRDEHVKRISASAYAALPESQRPVDLPQYDDTSPLPFELKPVIYFVEAEQAKLKGES

SEQ ID NO: 32 - protein, 441 aa, Ostreococcus tauri
MPDVLGPGDGDAYERVRSFHYDGFVVDDPEILPEALHDDVARAFDSLLREGEFTHDVLSAGNKVSRTFVTRTLLGDRGTTYHYQKLRLFAQPWDGEKRWEYATARRLNEALTRRTREILRGTRHGESECEYNVTLINRMDTREESEVALKDEALFDLGTTSVSWHSDSSLRENSTVAVYSTVDDPERADWSVALRALGKQCPALRVPLKDKATYYMCGDFNATHHHAVLTGSSARYSSTHRVGVVEKDTFQYIKRRCLEALALIPDLENKSASLDAKKIQLLAEIHREVEFQWIRMFHLQGDTHARQHKTYWTQRIAELTEAWDRMEACFRAILSKLKLSPESTPQPSRAYSMMLYAMKEVKELRDEHVKRISASAYAALPESQRPVDLPQYDDTSPLPFELKPVIYFVEAEQAKLKGESKRPAATKKAGQAKKKKRKVIK

SEQ ID NO: 33 - protein, 490 aa, Ostreococcus tauri
MKRTPTAEERERGAKKLRLLEELEDTWLPYLRKVIKPDVLGPGDGDAYERVRSFHYDGFVVDDPEILPEALHDDVARAFDSLLREGEFTHDVLSAGNKVSRTFVTRTLLGDRGTTYHYQKLRLFAQPWDGEKRWEYATARRLNEALTRRTREILRGTRHGESECEYNVTLINRMDTREESEVALKDEALFDLGTTSVSWHSDSSLRENSTVAVYSTVDDPERADWSVALRALGKQCPALRVPLKDKATYYMCGDFNATHHHAVLTGSSARYSSTHRVGVVEKDTFQYIKRRCLEALALIPDLENKSASLDAKKIQLLAEIHREVEFQWIRMFHLQGDTHARQHKTYWTQRIAELTEAWDRMEACFRAILSKLKLSPESTPQPSRAYSMMLYAMKEVKELRDEHVKRISASAYAALPESQRPVDLPQYDDTSPLPFELKPVIYFVEAEQAKLKGESRKVIKKRTPTAEERERGAKKLRLLEELEDTWLPYL

SEQ ID NO: 34 - protein, 791 aa, Ectocarpus sp
MRPRKTMTTATTVATTSRLLSPPTSEATTPIQHSNSGMEVSTEKTSHKKKRKSKRKRQQQERDTSSIPDASRQSRGSSSSSTRPPPPPPPPPPTTTTTTTSKKHSRIKEKPARFVHPHLDAELRRLGRSWLSPGDPLFKPALDRSYRGVRHEPGGSLPQAVHRGFRQSFDSLHEAGLFLYDTVQAGGKRLSRTFVTRTLVGDAGITYKYLGLRLFAHPWGLGESDFRKGPGDSLADALNDPCLADLFSNDGSGFDDNDRVADTLRKVGDLSEWMRLRAGAMLKEEVGEAGGERGSCAFNLTLINRMECSGAKRDLKPDPLFSMGKFSVSWHADSCLQDFSTIGVYHCTDPVPAEPDWGIALRVSTEARVGGGGGGSGDGDGYGVSNVEKTRRKEAERGVKPAGPKAIASVAASAAGAVPEKQGEQVLTPPLLIPLQSGDAYFLLDDFNHFHEHAVVSGSSTLRYSSTHRVADTDGNTFSHVQKRCERALAGGGSAAAGGDYHILNLAQVRAEQALLTELESEWLNQFWVQGRRHASLHPWWRGPMALVLATWRELERRTALTVRRLMSLRGQGGGEGVGPGGGGTAAETAGAEPAAIAKAFETVLRALEVRRESRSRWGARFADSAYRSLAADLAPVVPALWPAEGSSGGDVGEEGSPLLLPQSLGGIVSRLRECYTVVYRAASGGKKAGSAKAIAAGAASNWELFRAASSSSSSGGGGAGKKHGSALGKQQQQQQQQQQQQRKMRGLAGQDGLEKTKKRAGGVVKGGGDGGGGRTLKGQGSRRKDRVRER

SEQ ID NO: 35 - protein, 792 aa, Ectocarpus sp
MTMTTATTVATTSRLLSPPTSEATTPIQHSNSGMEVSTEKTSHKKKRKSKRKRQQQERDTSSIPDASRQSRGSSSSSTRPPPPPPPPPPTTTTTTTSKKHSRIKEKPARFVHPHLDAELRRLGRSWLSPGDPLFKPALDRSYRGVRHEPGGSLPQAVHRGFRQSFDSLHEAGLFLYDTVQAGGKRLSRTFVTRTLVGDAGITYKYLGLRLFAHPWGLGESDFRKGPGDSLADALNDPCLADLFSNDGSGFDDNDRVADTLRKVGDLSEWMRLRAGAMLKEEVGEAGGERGSCAFNLTLINRMECSGAKRDLKPDPLFSMGKFSVSWHADSCLQDFSTIGVYHCTDPVPAEPDWGIALRVSTEARVGGGGGGSGDGDGYGVSNVEKTRRKEAERGVKPAGPKAIASVAASAAGAVPEKQGEQVLTPPLLIPLQSGDAYFLLDDFNHFHEHAVVSGSSTLRYSSTHRVADTDGNTFSHVQKRCERALAGGGSAAAGGDYHILNLAQVRAEQALLTELESEWLNQFWVQGRRHASLHPWWRGPMALVLATWRELERRTALTVRRLMSLRGQGGGEGVGPGGGGTAAETAGAEPAAIAKAFETVLRALEVRRESRSRWGARFADSAYRSLAADLAPVVPALWPAEGSSGGDVGEEGSPLLLPQSLGGIVSRLRECYTVVYRAASGGKKAGSAKAIAAGAASNWELFRAASSSSSSGGGGAGKKHGSALGKQQQQQQQQQQQQRKMRGLAGQDGLEKTKKRAGGVVKGGGDGGGGRTLKGQGSRRKDRVRERRKVIK

SEQ ID NO: 36 - protein, 841 aa, Ectocarpus sp
MTLLLRETMNNLGVSDHAVLSRKTPQPYTMTTATTVATTSRLLSPPTSEATTPIQHSNSGMEVSTEKTSHKKKRKSKRKRQQQERDTSSIPDASRQSRGSSSSSTRPPPPPPPPPPTTTTTTTSKKHSRIKEKPARFVHPHLDAELRRLGRSWLSPGDPLFKPALDRSYRGVRHEPGGSLPQAVHRGFRQSFDSLHEAGLFLYDTVQAGGKRLSRTFVTRTLVGDAGITYKYLGLRLFAHPWGLGESDFRKGPGDSLADALNDPCLADLFSNDGSGFDDNDRVADTLRKVGDLSEWMRLRAGAMLKEEVGEAGGERGSCAFNLTLINRMECSGAKRDLKPDPLFSMGKFSVSWHADSCLQDFSTIGVYHCTDPVPAEPDWGIALRVSTEARVGGGGGGSGDGDGYGVSNVEKTRRKEAERGVKPAGPKAIASVAASAAGAVPEKQGEQVLTPPLLIPLQSGDAYFLLDDFNHFHEHAVVSGSSTLRYSSTHRVADTDGNTFSHVQKRCERALAGGGSAAAGGDYHILNLAQVRAEQALLTELESEWLNQFWVQGRRHASLHPWWRGPMALVLATWRELERRTALTVRRLMSLRGQGGGEGVGPGGGGTAAETAGAEPAAIAKAFETVLRALEVRRESRSRWGARFADSAYRSLAADLAPVVPALWPAEGSSGGDVGEEGSPLLLPQSLGGIVSRLRECYTVVYRAASGGKKAGSAKAIAAGAASNWELFRAASSSSSSGGGGAGKKHGSALGKQQQQQQQQQQQQRKMRGLAGQDGLEKTKKRAGGVVKGGGDGGGGRTLKGQGSRRKDRVRERTLLLRETMNNLGVSDHAVLSRKTPQPY

SEQ ID NO: 37 - protein, 722 aa, Conferva siliculosa
MPKKKRKVTTTSATTAARSRLPSPPTSAATTPIQHSNNGTEASPEKTSNKKKAKNKRKRQQECSIPAASQQSRGSSSSSTRPPPPTTTTLKKHSRIKEKPARFVHPHLDAELRRLGRSWLSPGDPLFTPALDRSYRGVRHEPAGSLPQAVHSGFRQSFDSLHEAGLFLYDTVQAGGKRLSRTFVTRTLVGDAGITYKYLGLRLFAHPWGLGESDFRKGPGDGLADALNDPCLADLFSKDGASSVRKSKDNLRGSRFDDNDRVADTLRKVGDLSEWMRLRAGAMLKEEVREAGGERGSCAFNLTLINRMECSGAKRDLKPDPLFSMGKCSVSWHADSCLQDFSTIGVYHCTDPVPAEPDWGIALRVSTEARVGGDGGGDGDGNGVSNDEKTRRKEAERGLKPAGPKAVASVAASAAEAVPEKQGEQVLTPPLLIPLQSGDAYFLLDDFNHFHEHAVVSGSSTLRYSSTHRVADTDGNTFSHVQKRCEQALAGGGSAAAGGDDQILNLAQVRAEQALLTELESEWLNQFWVQGRRHASLHPWWRGPMALVLATWRELERRTSLTVQHLMSLRGQDGGEALWPAEGSGGGDVGEEGSTLLLPQSLGGVISRLRECYTVVYRAASGGKKAGSAKAIAAGAASNWELFRAASSSASSGGGGAGKKHGSALGKQQQQQQQRKKRGAAGQDGLEKKKRAGGVVKGGGDGGGGRTSKGQRSRRKGRVRER

SEQ ID NO: 38 - protein, 721 aa, Conferva siliculosa
MTTTSATTAARSRLPSPPTSAATTPIQHSNNGTEASPEKTSNKKKAKNKRKRQQECSIPAASQQSRGSSSSSTRPPPPTTTTLKKHSRIKEKPARFVHPHLDAELRRLGRSWLSPGDPLFTPALDRSYRGVRHEPAGSLPQAVHSGFRQSFDSLHEAGLFLYDTVQAGGKRLSRTFVTRTLVGDAGITYKYLGLRLFAHPWGLGESDFRKGPGDGLADALNDPCLADLFSKDGASSVRKSKDNLRGSRFDDNDRVADTLRKVGDLSEWMRLRAGAMLKEEVREAGGERGSCAFNLTLINRMECSGAKRDLKPDPLFSMGKCSVSWHADSCLQDFSTIGVYHCTDPVPAEPDWGIALRVSTEARVGGDGGGDGDGNGVSNDEKTRRKEAERGLKPAGPKAVASVAASAAEAVPEKQGEQVLTPPLLIPLQSGDAYFLLDDFNHFHEHAVVSGSSTLRYSSTHRVADTDGNTFSHVQKRCEQALAGGGSAAAGGDDQILNLAQVRAEQALLTELESEWLNQFWVQGRRHASLHPWWRGPMALVLATWRELERRTSLTVQHLMSLRGQDGGEALWPAEGSGGGDVGEEGSTLLLPQSLGGVISRLRECYTVVYRAASGGKKAGSAKAIAAGAASNWELFRAASSSASSGGGGAGKKHGSALGKQQQQQQQRKKRGAAGQDGLEKKKRAGGVVKGGGDGGGGRTSKGQRSRRKGRVRERRNKKKK

SEQ ID NO: 39 - protein, 727 aa, Conferva siliculosa
MRNKKKKTTTSATTAARSRLPSPPTSAATTPIQHSNNGTEASPEKTSNKKKAKNKRKRQQECSIPAASQQSRGSSSSSTRPPPPTTTTLKKHSRIKEKPARFVHPHLDAELRRLGRSWLSPGDPLFTPALDRSYRGVRHEPAGSLPQAVHSGFRQSFDSLHEAGLFLYDTVQAGGKRLSRTFVTRTLVGDAGITYKYLGLRLFAHPWGLGESDFRKGPGDGLADALNDPCLADLFSKDGASSVRKSKDNLRGSRFDDNDRVADTLRKVGDLSEWMRLRAGAMLKEEVREAGGERGSCAFNLTLINRMECSGAKRDLKPDPLFSMGKCSVSWHADSCLQDFSTIGVYHCTDPVPAEPDWGIALRVSTEARVGGDGGGDGDGNGVSNDEKTRRKEAERGLKPAGPKAVASVAASAAEAVPEKQGEQVLTPPLLIPLQSGDAYFLLDDFNHFHEHAVVSGSSTLRYSSTHRVADTDGNTFSHVQKRCEQALAGGGSAAAGGDDQILNLAQVRAEQALLTELESEWLNQFWVQGRRHASLHPWWRGPMALVLATWRELERRTSLTVQHLMSLRGQDGGEALWPAEGSGGGDVGEEGSTLLLPQSLGGVISRLRECYTVVYRAASGGKKAGSAKAIAAGAASNWELFRAASSSASSGGGGAGKKHGSALGKQQQQQQQRKKRGAAGQDGLEKKKRAGGVVKGGGDGGGGRTSKGQRSRRKGRVRERRNKKKK

SEQ ID NO: 40 - protein, 440 aa, Fragilariopsis cylindrus
MKRPAATKKAGQAKKKKPKKKRKVLTPEDGVYFQKHLQDHYKGFVHLPVDRLEPRDFHEEFKNSLERLRDAGYYQYDVVMAGGKYSSRTFVKRTLVGNPGITYKYLGLRLFAHAWSGPGCTPLMKSIGDMNQSMIKMTEQFPENERCDYNLTLINYMEPTTHTKVGFKDEANYGMGKVSVSWHADSSLVDNSSIGVYHCLPTQRNSKWDWKIALRPLAIESKDNTGSTKRDNKSTTPKPVVVNTKDGDAYFLLGNFNMKHQHCVLAGSQANRISSTHRVAVTIEDTYDYILKRVKIARKRFRLQMETIPPSLQSPVVGLDAKVIRYCQRILTEVEMEWIAQYWLQGDQHDKMRVWWQKPMKTLEAYWCALEVYTYRLFEFLLSRIASNDTVPIDVVKVLIIEFKTRQSFREQWDERRSDKIYQRRVSEEFRPVARPIFEN

SEQ ID NO: 41 - protein, 451 aa, Fragilariopsis cylindrus
MLTPEDGVYFQKHLQDHYKGFVHLPVDRLEPRDFHEEFKNSLERLRDAGYYQYDVVMAGGKYSSRTFVKRTLVGNPGITYKYLGLRLFAHAWSGPGCTPLMKSIGDMNQSMIKMTEQFPENERCDYNLTLINYMEPTTHTKVGFKDEANYGMGKVSVSWHADSSLVDNSSIGVYHCLPTQRNSKWDWKIALRPLAIESKDNTGSTKRDNKSTTPKPVVVNTKDGDAYFLLGNFNMKHQHCVLAGSQANRISSTHRVAVTIEDTYDYILKRVKIARKRFRLQMETIPPSLQSPVVGLDAKVIRYCQRILTEVEMEWIAQYWLQGDQHDKMRVWWQKPMKTLEAYWCALEVYTYRLFEFLLSRIASNDTVPIDVVKVLIIEFKTRQSFREQWDERRSDKIYQRRVSEEFRPVARPIFENKRTPTAEERERGAKKLRLLEELEDTWLPYLRPRK

SEQ ID NO: 42 - protein, 461 aa, Fragilariopsis cylindrus
MRNKKKKKRPAATKKAGQAKKKKLTPEDGVYFQKHLQDHYKGFVHLPVDRLEPRDFHEEFKNSLERLRDAGYYQYDVVMAGGKYSSRTFVKRTLVGNPGITYKYLGLRLFAHAWSGPGCTPLMKSIGDMNQSMIKMTEQFPENERCDYNLTLINYMEPTTHTKVGFKDEANYGMGKVSVSWHADSSLVDNSSIGVYHCLPTQRNSKWDWKIALRPLAIESKDNTGSTKRDNKSTTPKPVVVNTKDGDAYFLLGNFNMKHQHCVLAGSQANRISSTHRVAVTIEDTYDYILKRVKIARKRFRLQMETIPPSLQSPVVGLDAKVIRYCQRILTEVEMEWIAQYWLQGDQHDKMRVWWQKPMKTLEAYWCALEVYTYRLFEFLLSRIASNDTVPIDVVKVLIIEFKTRQSFREQWDERRSDKIYQRRVSEEFRPVARPIFENKRPAATKKAGQAKKKKRNKKKK

SEQ ID NO: 43 - protein, 555 aa, Acanthaster planci
MTLLLRETMNNLGVSDHAVLSRKTPQPYRFLSLNVLRRWMSKMSKRRQTEDLGKEVKKKKLLSEVARGRLQFLMPDHPDFKSLMRKSYFNFAHEPSTGIPVSLHEELTWALDILRYHGYFYRDWVKVKGQTVQTPISRTLIGEPGTTYKYLGLRLFTIPWSFGHHKPESEVELASETIGKLNEHYKAVSRRLLRKKTAEQTHLKSSPSQEVAPCSSKDRPRERICVEEPKQMTHGLSIEEGTNFNVVLINYMDPEDPDLRLKPEPYYGMGPLAVSWHMDGNLVRGSTVAVYNHTCSSDGGDSTTDSDWMVGFKVSWDIETPGVAIPLQTGESYFMLGDLNDTHQHCVVAGSQARFSTTHRVADCQQGTLSYIQQRCLEALGNLSQLENGEYELKSFQAGHLDFTETVHNEVEFEWLRQFWMQGSRHAAERGGWVPAMECLEADWNKMEHMTKLAVEEANRLGPEEGSVIAEALLPHLKERRKLRQECLDKFPRRLLETIHRDFLPIHRPKWDNDDPSQPLPFDLKGIIRKMRLLCNGKRIKSPSDSESSDTGLHS

SEQ ID NO: 44 - protein, 533 aa, Acanthaster planci
MRFLSLNVLRRWMSKMSKRRQTEDLGKEVKKKKLLSEVARGRLQFLMPDHPDFKSLMRKSYFNFAHEPSTGIPVSLHEELTWALDILRYHGYFYRDWVKVKGQTVQTPISRTLIGEPGTTYKYLGLRLFTIPWSFGHHKPESEVELASETIGKLNEHYKAVSRRLLRKKTAEQTHLKSSPSQEVAPCSSKDRPRERICVEEPKQMTHGLSIEEGTNFNVVLINYMDPEDPDLRLKPEPYYGMGPLAVSWHMDGNLVRGSTVAVYNHTCSSDGGDSTTDSDWMVGFKVSWDIETPGVAIPLQTGESYFMLGDLNDTHQHCVVAGSQARFSTTHRVADCQQGTLSYIQQRCLEALGNLSQLENGEYELKSFQAGHLDFTETVHNEVEFEWLRQFWMQGSRHAAERGGWVPAMECLEADWNKMEHMTKLAVEEANRLGPEEGSVIAEALLPHLKERRKLRQECLDKFPRRLLETIHRDFLPIHRPKWDNDDPSQPLPFDLKGIIRKMRLLCNGKRIKSPSDSESSDTGLHSRKVIK

SEQ ID NO: 45 - protein, 538 aa, Acanthaster planci
MRKVIKRFLSLNVLRRWMSKMSKRRQTEDLGKEVKKKKLLSEVARGRLQFLMPDHPDFKSLMRKSYFNFAHEPSTGIPVSLHEELTWALDILRYHGYFYRDWVKVKGQTVQTPISRTLIGEPGTTYKYLGLRLFTIPWSFGHHKPESEVELASETIGKLNEHYKAVSRRLLRKKTAEQTHLKSSPSQEVAPCSSKDRPRERICVEEPKQMTHGLSIEEGTNFNVVLINYMDPEDPDLRLKPEPYYGMGPLAVSWHMDGNLVRGSTVAVYNHTCSSDGGDSTTDSDWMVGFKVSWDIETPGVAIPLQTGESYFMLGDLNDTHQHCVVAGSQARFSTTHRVADCQQGTLSYIQQRCLEALGNLSQLENGEYELKSFQAGHLDFTETVHNEVEFEWLRQFWMQGSRHAAERGGWVPAMECLEADWNKMEHMTKLAVEEANRLGPEEGSVIAEALLPHLKERRKLRQECLDKFPRRLLETIHRDFLPIHRPKWDNDDPSQPLPFDLKGIIRKMRLLCNGKRIKSPSDSESSDTGLHSRKVIK

SEQ ID NO: 46 - protein, 489 aa, Saccoglossus kowalevskii
MRPRKNPRMKRKIPRIPLVTSEGEVAGQLALPIRKQKLLSAVKETQVKFLSPVDTDYKALVAENYDNFVVQPGTELSSELHTRLQQGFETLLTNGYLYQHRIRFRNKTVMTPVSRTLIGEPGMTYRYLNLRLFALPWTFDDKKKLSDVEKACNAFYELNTYFKDHVNKLITEKFASSTGRKIDETDDSLKTIIQRNTEFKATILNYMDPSEIRLKQEPYYNMGDIAVSWHKDESLVDGSTVAVYNHVPMEARQDCSKWKVGLKVAWDITTPAVCTPLNNKDCYYMLDTMNDTHQHCVIAGTLPRYSSTHRVVESSDSTLCYIQQRCQTALDNIGYKDQIPYLKSLETDVLQLIEEIHSEIEFEWLRQFWMQGTQHSQERQYWLKPMEQLQEDWKTMELMTKLMIDIVVKKKDQSHMIAKILLPSLVERNELRNEWMNRYSEKEFYHIPEEHRPIYEPCWTDANSEMPLPFDLSQHIDIIQECMDTNDSQ

SEQ ID NO: 47 - protein, 491 aa, Saccoglossus kowalevskii
MNPRMKRKIPRIPLVTSEGEVAGQLALPIRKQKLLSAVKETQVKFLSPVDTDYKALVAENYDNFVVQPGTELSSELHTRLQQGFETLLTNGYLYQHRIRFRNKTVMTPVSRTLIGEPGMTYRYLNLRLFALPWTFDDKKKLSDVEKACNAFYELNTYFKDHVNKLITEKFASSTGRKIDETDDSLKTIIQRNTEFKATILNYMDPSEIRLKQEPYYNMGDIAVSWHKDESLVDGSTVAVYNHVPMEARQDCSKWKVGLKVAWDITTPAVCTPLNNKDCYYMLDTMNDTHQHCVIAGTLPRYSSTHRVVESSDSTLCYIQQRCQTALDNIGYKDQIPYLKSLETDVLQLIEEIHSEIEFEWLRQFWMQGTQHSQERQYWLKPMEQLQEDWKTMELMTKLMIDIVVKKKDQSHMIAKILLPSLVERNELRNEWMNRYSEKEFYHIPEEHRPIYEPCWTDANSEMPLPFDLSQHIDIIQECMDTNDSQRNKKKK

SEQ ID NO: 48 - protein, 545 aa, Saccoglossus kowalevskii
MKRTPTAEERERGAKKLRLLEELEDTWLPYLNPRMKRKIPRIPLVTSEGEVAGQLALPIRKQKLLSAVKETQVKFLSPVDTDYKALVAENYDNFVVQPGTELSSELHTRLQQGFETLLTNGYLYQHRIRFRNKTVMTPVSRTLIGEPGMTYRYLNLRLFALPWTFDDKKKLSDVEKACNAFYELNTYFKDHVNKLITEKFASSTGRKIDETDDSLKTIIQRNTEFKATILNYMDPSEIRLKQEPYYNMGDIAVSWHKDESLVDGSTVAVYNHVPMEARQDCSKWKVGLKVAWDITTPAVCTPLNNKDCYYMLDTMNDTHQHCVIAGTLPRYSSTHRVVESSDSTLCYIQQRCQTALDNIGYKDQIPYLKSLETDVLQLIEEIHSEIEFEWLRQFWMQGTQHSQERQYWLKPMEQLQEDWKTMELMTKLMIDIVVKKKDQSHMIAKILLPSLVERNELRNEWMNRYSEKEFYHIPEEHRPIYEPCWTDANSEMPLPFDLSQHIDIIQECMDTNDSQKRTPTAEERERGAKKLRLLEELEDTWLPYL